European Patent Specification EP 3 647 320 B1, published October 9, 2024. Title: PEPTIDE FOR BINDING TO ACETYLCHOLINE RECEPTORS. Applicant: KOREA INSTITUTE OF CERAMIC ENGINEERING & TECHNOLOGY. The sequence listing filed with the application follows.

SEQUENCE LISTING (31 sequences)

SEQ ID NO: 1 - protein, 6 aa, Artificial Sequence
  Ach-R
KGTLNR

SEQ ID NO: 2 - protein, 6 aa, Artificial Sequence
  Ach-R
RKSLLR

SEQ ID NO: 3 - protein, 6 aa, Artificial Sequence
  Ach-R
EDKGKN

SEQ ID NO: 4 - protein, 6 aa, Artificial Sequence
  Ach-R
RDKLQM

SEQ ID NO: 5 - protein, 6 aa, Artificial Sequence
  Ach-R
QLGQLS

SEQ ID NO: 6 - protein, 6 aa, Artificial Sequence
  Ach-R
GRLSAS

SEQ ID NO: 7 - protein, 6 aa, Artificial Sequence
  Ach-R
RQLNNQ

SEQ ID NO: 8 - protein, 6 aa, Artificial Sequence
  Ach-R
DNLQNN

SEQ ID NO: 9 - protein, 6 aa, Artificial Sequence
  Ach-R
LYQRLG

SEQ ID NO: 10 - protein, 6 aa, Artificial Sequence
  Ach-R
NKQVKF

SEQ ID NO: 11 - protein, 6 aa, Artificial Sequence
  Ach-R
ETYDSK

SEQ ID NO: 12 - protein, 11 aa, Artificial Sequence
  Ach-R
WTWKGKGTLNR

SEQ ID NO: 13 - protein, 11 aa, Artificial Sequence
  Ach-R
WTWKGKGTLNR

SEQ ID NO: 14 - protein, 11 aa, Artificial Sequence
  Ach-R
WTWKGEDKGKN

SEQ ID NO: 15 - protein, 11 aa, Artificial Sequence
  Ach-R
WTWKGRDKLQM

SEQ ID NO: 16 - protein, 11 aa, Artificial Sequence
  Ach-R
WTWKGQLGQLS

SEQ ID NO: 17 - protein, 11 aa, Artificial Sequence
  Ach-R
WTWKGGRLSAS

SEQ ID NO: 18 - protein, 11 aa, Artificial Sequence
  Ach-R
WTWKGRQLNNQ

SEQ ID NO: 19 - protein, 11 aa, Artificial Sequence
  Ach-R
WTWKGDNLQNN

SEQ ID NO: 20 - protein, 11 aa, Artificial Sequence
  Ach-R
WTWKGLYQRLG

SEQ ID NO: 21 - protein, 11 aa, Artificial Sequence
  Ach-R
WTWKGNKQVKF

SEQ ID NO: 22 - protein, 11 aa, Artificial Sequence
  Ach-R
WTWKGETYDSK

SEQ ID NO: 23 - protein, 11 aa, Artificial Sequence
  Ach-R
WTWKGKGTLNR

SEQ ID NO: 24 - protein, 11 aa, Artificial Sequence
  Ach-R
WTWKGRKSLLR

SEQ ID NO: 25 - protein, 11 aa, Artificial Sequence
  Ach-R
WTWKGEDKGKN

SEQ ID NO: 26 - protein, 11 aa, Artificial Sequence
  Ach-R
WTWKGRDKLQM

SEQ ID NO: 27 - protein, 10 aa, Artificial Sequence
  Ach-R
TWKGKGTLNR

SEQ ID NO: 28 - protein, 9 aa, Artificial Sequence
  Ach-R
WKGKGTLNR

SEQ ID NO: 29 - protein, 10 aa, Artificial Sequence
  Ach-R
WTWKGKGTLN

SEQ ID NO: 30 - protein, 9 aa, Artificial Sequence
  Ach-R
WTWKGKGTL

SEQ ID NO: 31 - protein, 6 aa, Artificial Sequence
  Ach-R
KGTLNR